European Patent Specification EP 3 561 055 B1, published September 30, 2026. Title: Modified polypeptide with attenuated activity of citrate synthase and a method for producing L-amino acid using the same. Applicant: CJ CheilJedang Corporation. The sequence listing filed with the application follows.

SEQUENCE LISTING (62 sequences)

SEQ ID NO: 1 - protein, 437 aa, Corynebacterium glutamicum [sequence omitted]

SEQ ID NO: 2 - DNA, 1314 bp, Corynebacterium glutamicum
  gene (1)..(1314): gltA
atgtttgaaagggatatcgtggctactgataacaacaaggctgtcctgcactaccccggtggcgagttcgaaatggacatcatcgaggcttctgagggtaacaacggtgttgtcctgggcaagatgctgtctgagactggactgatcacttttgacccaggttatgtgagcactggctccaccgagtcgaagatcacctacatcgatggcgatgcgggaatcctgcgttaccgcggctatgacatcgctgatctggctgagaatgccaccttcaacgaggtttcttacctacttatcaacggtgagctaccaaccccagatgagcttcacaagtttaacgacgagattcgccaccacacccttctggacgaggacttcaagtcccagttcaacgtgttcccacgcgacgctcacccaatggcaaccttggcttcctcggttaacattttgtctacctactaccaggaccagctgaacccactcgatgaggcacagcttgataaggcaaccgttcgcctcatggcaaaggttccaatgctggctgcgtacgcacaccgcgcacgcaagggtgctccttacatgtacccagacaactccctcaatgcgcgtgagaacttcctgcgcatgatgttcggttacccaaccgagccatacgagatcgacccaatcatggtcaaggctctggacaagctgctcatcctgcacgctgaccacgagcagaactgctccacctccaccgttcgtatgatcggttccgcacaggccaacatgtttgtctccatcgctggtggcatcaacgctctgtccggcccactgcacggtggcgcaaaccaggctgttctggagatgctcgaagacatcaagagcaaccacggtggcgacgcaaccgagttcatgaacaaggtcaagaacaaggaagacggcgtccgcctcatgggcttcggacaccgcgtttacaagaactacgatccacgtgcagcaatcgtcaaggagaccgcacacgagatcctcgagcacctcggtggcgacgatcttctggatctggcaatcaagctggaagaaattgcactggctgatgattacttcatctcccgcaagctctacccgaacgtagacttctacaccggcctgatctaccgcgcaatgggcttcccaactgacttcttcaccgtattgttcgcaatcggtcgtctgccaggatggatcgctcactaccgcgagcagctcggtgcagcaggcaacaagatcaaccgcccacgccaggtctacaccggcaacgaatcccgcaagttggttcctcgcgaggagcgctaa

SEQ ID NO: 3 - protein, 437 aa, Unknown
  N241T
MFERDIVATDNNKAVLHYPGGEFEMDIIEASEGNNGVVLGKMLSETGLITFDPGYVSTGSTESKITYIDGDAGILRYRGYDIADLAENATFNEVSYLLINGELPTPDELHKFNDEIRHHTLLDEDFKSQFNVFPRDAHPMATLASSVNILSTYYQDQLNPLDEAQLDKATVRLMAKVPMLAAYAHRARKGAPYMYPDNSLNARENFLRMMFGYPTEPYEIDPIMVKALDKLLILHADHEQTCSTSTVRMIGSAQANMFVSIAGGINALSGPLHGGANQAVLEMLEDIKSNHGGDATEFMNKVKNKEDGVRLMGFGHRVYKNYDPRAAIVKETAHEILEHLGGDDLLDLAIKLEEIALADDYFISRKLYPNVDFYTGLIYRAMGFPTDFFTVLFAIGRLPGWIAHYREQLGAAGNKINRPRQVYTGNESRKLVPREER

SEQ ID NO: 4 - DNA, 1314 bp, Unknown
  N241T
atgtttgaaagggatatcgtggctactgataacaacaaggctgtcctgcactaccccggtggcgagttcgaaatggacatcatcgaggcttctgagggtaacaacggtgttgtcctgggcaagatgctgtctgagactggactgatcacttttgacccaggttatgtgagcactggctccaccgagtcgaagatcacctacatcgatggcgatgcgggaatcctgcgttaccgcggctatgacatcgctgatctggctgagaatgccaccttcaacgaggtttcttacctacttatcaacggtgagctaccaaccccagatgagcttcacaagtttaacgacgagattcgccaccacacccttctggacgaggacttcaagtcccagttcaacgtgttcccacgcgacgctcacccaatggcaaccttggcttcctcggttaacattttgtctacctactaccaggaccagctgaacccactcgatgaggcacagcttgataaggcaaccgttcgcctcatggcaaaggttccaatgctggctgcgtacgcacaccgcgcacgcaagggtgctccttacatgtacccagacaactccctcaatgcgcgtgagaacttcctgcgcatgatgttcggttacccaaccgagccatacgagatcgacccaatcatggtcaaggctctggacaagctgctcatcctgcacgctgaccacgagcagacctgctccacctccaccgttcgtatgatcggttccgcacaggccaacatgtttgtctccatcgctggtggcatcaacgctctgtccggcccactgcacggtggcgcaaaccaggctgttctggagatgctcgaagacatcaagagcaaccacggtggcgacgcaaccgagttcatgaacaaggtcaagaacaaggaagacggcgtccgcctcatgggcttcggacaccgcgtttacaagaactacgatccacgtgcagcaatcgtcaaggagaccgcacacgagatcctcgagcacctcggtggcgacgatcttctggatctggcaatcaagctggaagaaattgcactggctgatgattacttcatctcccgcaagctctacccgaacgtagacttctacaccggcctgatctaccgcgcaatgggcttcccaactgacttcttcaccgtattgttcgcaatcggtcgtctgccaggatggatcgctcactaccgcgagcagctcggtgcagcaggcaacaagatcaaccgcccacgccaggtctacaccggcaacgaatcccgcaagttggttcctcgcgaggagcgctaa

SEQ ID NO: 5 - DNA, 21 bp, Artificial Sequence
  primer
atgtttgaaagggatatcgtg

SEQ ID NO: 6 - DNA, 21 bp, Artificial Sequence
  primer
ttagcgctcctcgcgaggaac

SEQ ID NO: 7 - DNA, 30 bp, Artificial Sequence
  primer
cggggatcctctagacgatgaaaaacgccc

SEQ ID NO: 8 - DNA, 30 bp, Artificial Sequence
  primer
caggtcgactctagactgcacgtggatcgt

SEQ ID NO: 9 - DNA, 24 bp, Artificial Sequence
  primer
actgggactatttgttcggaaaaa

SEQ ID NO: 10 - DNA, 24 bp, Artificial Sequence
  primer
cgaacaaatagtcccagttcaacg

SEQ ID NO: 11 - DNA, 35 bp, Artificial Sequence
  primer
cggggatcctctagaagatgctgtctgagactgga

SEQ ID NO: 12 - DNA, 35 bp, Artificial Sequence
  primer
caggtcgactctagacgctaaatttagcgctcctc

SEQ ID NO: 13 - DNA, 30 bp, Artificial Sequence
  primer
ggaggtggagcatgcctgctcgtggtcagc

SEQ ID NO: 14 - DNA, 30 bp, Artificial Sequence
  primer
gaccacgagcaggcatgctccacctccacc

SEQ ID NO: 15 - DNA, 30 bp, Artificial Sequence
  primer
ggaggtggagcagacctgctcgtggtcagc

SEQ ID NO: 16 - DNA, 30 bp, Artificial Sequence
  primer
gaccacgagcaggtctgctccacctccacc

SEQ ID NO: 17 - DNA, 30 bp, Artificial Sequence
  primer
ggaggtggagcactgctgctcgtggtcagc

SEQ ID NO: 18 - DNA, 30 bp, Artificial Sequence
  primer
gaccacgagcagcagtgctccacctccacc

SEQ ID NO: 19 - DNA, 30 bp, Artificial Sequence
  primer
ggaggtggagcagtgctgctcgtggtcagc

SEQ ID NO: 20 - DNA, 30 bp, Artificial Sequence
  primer
gaccacgagcagcactgctccacctccacc

SEQ ID NO: 21 - DNA, 30 bp, Artificial Sequence
  primer
ggaggtggagcagcgctgctcgtggtcagc

SEQ ID NO: 22 - DNA, 30 bp, Artificial Sequence
  primer
gaccacgagcagcgctgctccacctccacc

SEQ ID NO: 23 - DNA, 30 bp, Artificial Sequence
  primer
ggaggtggagcatggctgctcgtggtcagc

SEQ ID NO: 24 - DNA, 30 bp, Artificial Sequence
  primer
gaccacgagcagccatgctccacctccacc

SEQ ID NO: 25 - DNA, 30 bp, Artificial Sequence
  primer
ggaggtggagcacagctgctcgtggtcagc

SEQ ID NO: 26 - DNA, 30 bp, Artificial Sequence
  primer
gaccacgagcagctgtgctccacctccacc

SEQ ID NO: 27 - DNA, 30 bp, Artificial Sequence
  primer
ggaggtggagcagtactgctcgtggtcagc

SEQ ID NO: 28 - DNA, 30 bp, Artificial Sequence
  primer
gaccacgagcagtactgctccacctccacc

SEQ ID NO: 29 - DNA, 30 bp, Artificial Sequence
  primer
ggaggtggagcaggactgctcgtggtcagc

SEQ ID NO: 30 - DNA, 30 bp, Artificial Sequence
  primer
gaccacgagcagtcctgctccacctccacc

SEQ ID NO: 31 - DNA, 30 bp, Artificial Sequence
  primer
ggaggtggagcacttctgctcgtggtcagc

SEQ ID NO: 32 - DNA, 30 bp, Artificial Sequence
  primer
gaccacgagcagaagtgctccacctccacc

SEQ ID NO: 33 - DNA, 30 bp, Artificial Sequence
  primer
ggaggtggagcacatctgctcgtggtcagc

SEQ ID NO: 34 - DNA, 30 bp, Artificial Sequence
  primer
gaccacgagcagatgtgctccacctccacc

SEQ ID NO: 35 - DNA, 30 bp, Artificial Sequence
  primer
ggaggtggagcagatctgctcgtggtcagc

SEQ ID NO: 36 - DNA, 30 bp, Artificial Sequence
  primer
gaccacgagcagatctgctccacctccacc

SEQ ID NO: 37 - DNA, 30 bp, Artificial Sequence
  primer
ggaggtggagcattcctgctcgtggtcagc

SEQ ID NO: 38 - DNA, 30 bp, Artificial Sequence
  primer
gaccacgagcaggaatgctccacctccacc

SEQ ID NO: 39 - DNA, 30 bp, Artificial Sequence
  primer
ggaggtggagcagtcctgctcgtggtcagc

SEQ ID NO: 40 - DNA, 30 bp, Artificial Sequence
  primer
gaccacgagcaggactgctccacctccacc

SEQ ID NO: 41 - DNA, 30 bp, Artificial Sequence
  primer
ggaggtggagcagccctgctcgtggtcagc

SEQ ID NO: 42 - DNA, 30 bp, Artificial Sequence
  primer
gaccacgagcagggctgctccacctccacc

SEQ ID NO: 43 - DNA, 30 bp, Artificial Sequence
  primer
ggaggtggagcagcactgctcgtggtcagc

SEQ ID NO: 44 - DNA, 30 bp, Artificial Sequence
  primer
gaccacgagcagtggtgctccacctccacc

SEQ ID NO: 45 - DNA, 30 bp, Artificial Sequence; identical to SEQ ID NO: 43
  primer

SEQ ID NO: 46 - DNA, 30 bp, Artificial Sequence
  primer
gaccacgagcagtgctgctccacctccacc

SEQ ID NO: 47 - DNA, 30 bp, Artificial Sequence
  primer
ggaggtggagcagaactgctcgtggtcagc

SEQ ID NO: 48 - DNA, 30 bp, Artificial Sequence
  primer
gaccacgagcagttctgctccacctccacc

SEQ ID NO: 49 - DNA, 30 bp, Artificial Sequence
  primer
ggaggtggagcaggtctgctcgtggtcagc

SEQ ID NO: 50 - DNA, 30 bp, Artificial Sequence
  primer
gaccacgagcagacctgctccacctccacc

SEQ ID NO: 51 - DNA, 29 bp, Artificial Sequence
  primer
tcctctagactggtcgcctgatgttctac

SEQ ID NO: 52 - DNA, 29 bp, Artificial Sequence
  primer
gactctagattagtccctttcgaggcgga

SEQ ID NO: 53 - DNA, 20 bp, Artificial Sequence
  primer
gccaaaacctccacgcgatc

SEQ ID NO: 54 - DNA, 20 bp, Artificial Sequence
  primer
atcgcgtggaggttttggct

SEQ ID NO: 55 - DNA, 28 bp, Artificial Sequence
  primer
acggatcccagactccaaagcaaaagcg

SEQ ID NO: 56 - DNA, 28 bp, Artificial Sequence
  primer
acggatccaaccaaacttgctcacactc

SEQ ID NO: 57 - DNA, 30 bp, Artificial Sequence
  primer
acaccacggcagaaccaggtgcaaaggaca

SEQ ID NO: 58 - DNA, 30 bp, Artificial Sequence
  primer
ctggttctgccgtggtgtgcatcatctctg

SEQ ID NO: 59 - protein, 437 aa, Unknown
  N241S
MFERDIVATDNNKAVLHYPGGEFEMDIIEASEGNNGVVLGKMLSETGLITFDPGYVSTGSTESKITYIDGDAGILRYRGYDIADLAENATFNEVSYLLINGELPTPDELHKFNDEIRHHTLLDEDFKSQFNVFPRDAHPMATLASSVNILSTYYQDQLNPLDEAQLDKATVRLMAKVPMLAAYAHRARKGAPYMYPDNSLNARENFLRMMFGYPTEPYEIDPIMVKALDKLLILHADHEQSCSTSTVRMIGSAQANMFVSIAGGINALSGPLHGGANQAVLEMLEDIKSNHGGDATEFMNKVKNKEDGVRLMGFGHRVYKNYDPRAAIVKETAHEILEHLGGDDLLDLAIKLEEIALADDYFISRKLYPNVDFYTGLIYRAMGFPTDFFTVLFAIGRLPGWIAHYREQLGAAGNKINRPRQVYTGNESRKLVPREER

SEQ ID NO: 60 - DNA, 1314 bp, Unknown
  N241S
atgtttgaaagggatatcgtggctactgataacaacaaggctgtcctgcactaccccggtggcgagttcgaaatggacatcatcgaggcttctgagggtaacaacggtgttgtcctgggcaagatgctgtctgagactggactgatcacttttgacccaggttatgtgagcactggctccaccgagtcgaagatcacctacatcgatggcgatgcgggaatcctgcgttaccgcggctatgacatcgctgatctggctgagaatgccaccttcaacgaggtttcttacctacttatcaacggtgagctaccaaccccagatgagcttcacaagtttaacgacgagattcgccaccacacccttctggacgaggacttcaagtcccagttcaacgtgttcccacgcgacgctcacccaatggcaaccttggcttcctcggttaacattttgtctacctactaccaggaccagctgaacccactcgatgaggcacagcttgataaggcaaccgttcgcctcatggcaaaggttccaatgctggctgcgtacgcacaccgcgcacgcaagggtgctccttacatgtacccagacaactccctcaatgcgcgtgagaacttcctgcgcatgatgttcggttacccaaccgagccatacgagatcgacccaatcatggtcaaggctctggacaagctgctcatcctgcacgctgaccacgagcagtcctgctccacctccaccgttcgtatgatcggttccgcacaggccaacatgtttgtctccatcgctggtggcatcaacgctctgtccggcccactgcacggtggcgcaaaccaggctgttctggagatgctcgaagacatcaagagcaaccacggtggcgacgcaaccgagttcatgaacaaggtcaagaacaaggaagacggcgtccgcctcatgggcttcggacaccgcgtttacaagaactacgatccacgtgcagcaatcgtcaaggagaccgcacacgagatcctcgagcacctcggtggcgacgatcttctggatctggcaatcaagctggaagaaattgcactggctgatgattacttcatctcccgcaagctctacccgaacgtagacttctacaccggcctgatctaccgcgcaatgggcttcccaactgacttcttcaccgtattgttcgcaatcggtcgtctgccaggatggatcgctcactaccgcgagcagctcggtgcagcaggcaacaagatcaaccgcccacgccaggtctacaccggcaacgaatcccgcaagttggttcctcgcgaggagcgctaa

SEQ ID NO: 61 - protein, 437 aa, Unknown
  N241Y
MFERDIVATDNNKAVLHYPGGEFEMDIIEASEGNNGVVLGKMLSETGLITFDPGYVSTGSTESKITYIDGDAGILRYRGYDIADLAENATFNEVSYLLINGELPTPDELHKFNDEIRHHTLLDEDFKSQFNVFPRDAHPMATLASSVNILSTYYQDQLNPLDEAQLDKATVRLMAKVPMLAAYAHRARKGAPYMYPDNSLNARENFLRMMFGYPTEPYEIDPIMVKALDKLLILHADHEQYCSTSTVRMIGSAQANMFVSIAGGINALSGPLHGGANQAVLEMLEDIKSNHGGDATEFMNKVKNKEDGVRLMGFGHRVYKNYDPRAAIVKETAHEILEHLGGDDLLDLAIKLEEIALADDYFISRKLYPNVDFYTGLIYRAMGFPTDFFTVLFAIGRLPGWIAHYREQLGAAGNKINRPRQVYTGNESRKLVPREER

SEQ ID NO: 62 - DNA, 1314 bp, Unknown
  N241Y
atgtttgaaagggatatcgtggctactgataacaacaaggctgtcctgcactaccccggtggcgagttcgaaatggacatcatcgaggcttctgagggtaacaacggtgttgtcctgggcaagatgctgtctgagactggactgatcacttttgacccaggttatgtgagcactggctccaccgagtcgaagatcacctacatcgatggcgatgcgggaatcctgcgttaccgcggctatgacatcgctgatctggctgagaatgccaccttcaacgaggtttcttacctacttatcaacggtgagctaccaaccccagatgagcttcacaagtttaacgacgagattcgccaccacacccttctggacgaggacttcaagtcccagttcaacgtgttcccacgcgacgctcacccaatggcaaccttggcttcctcggttaacattttgtctacctactaccaggaccagctgaacccactcgatgaggcacagcttgataaggcaaccgttcgcctcatggcaaaggttccaatgctggctgcgtacgcacaccgcgcacgcaagggtgctccttacatgtacccagacaactccctcaatgcgcgtgagaacttcctgcgcatgatgttcggttacccaaccgagccatacgagatcgacccaatcatggtcaaggctctggacaagctgctcatcctgcacgctgaccacgagcagtactgctccacctccaccgttcgtatgatcggttccgcacaggccaacatgtttgtctccatcgctggtggcatcaacgctctgtccggcccactgcacggtggcgcaaaccaggctgttctggagatgctcgaagacatcaagagcaaccacggtggcgacgcaaccgagttcatgaacaaggtcaagaacaaggaagacggcgtccgcctcatgggcttcggacaccgcgtttacaagaactacgatccacgtgcagcaatcgtcaaggagaccgcacacgagatcctcgagcacctcggtggcgacgatcttctggatctggcaatcaagctggaagaaattgcactggctgatgattacttcatctcccgcaagctctacccgaacgtagacttctacaccggcctgatctaccgcgcaatgggcttcccaactgacttcttcaccgtattgttcgcaatcggtcgtctgccaggatggatcgctcactaccgcgagcagctcggtgcagcaggcaacaagatcaaccgcccacgccaggtctacaccggcaacgaatcccgcaagttggttcctcgcgaggagcgctaa